European Patent Application EP 4 663 202 A1, published December 17, 2025. Title: PHARMACEUTICAL PREPARATION CONTAINING ANTI-VEGFA/VEGFC BISPECIFIC BINDING PROTEIN. Applicant: INNOVENT BIOLOGICS (SUZHOU) CO., LTD. The sequence listing filed with the application follows.

SEQUENCE LISTING (10 sequences)

SEQ ID NO: 1 - protein, 10 aa, synthetic construct
  source 1..10: note; note (original language) = CDR1 sequence
GSSFSPYAMG

SEQ ID NO: 2 - protein, 16 aa, synthetic construct
  source 1..16: note; note (original language) = CDR2 sequence
ATSSGGFTLYADSVKG

SEQ ID NO: 3 - protein, 10 aa, synthetic construct
  source 1..10: note; note (original language) = CDR3 sequence
YYREYDPEMY

SEQ ID NO: 4 - protein, 118 aa, synthetic construct
  source 1..118: note; note (original language) = VHH sequence
EVQLVESGGGLVQPGGSLRLSCAASGSSFSPYAMGWYRQAPGKQRELVSATSSGGFTLYADSVKGRFTISRDNSKNTVYLQMNSLRAEDTAVYYCYTYYREYDPEMYWGQGTQVTVSS

SEQ ID NO: 5 - protein, 431 aa, synthetic construct
  source 1..431: note; note (original language) = Fc fusion protein of VEGFA binding domain
SDTGRPFVEMYSEIPEIIHMTEGRELVIPCRVTSPNITVTLKKFPLDTLIPDGKRIIWDSRKGFIISNATYKEIGLLTCEATVNGHLYKTNYLTHRQTNTIIDVVLSPSHGIELSVGEKLVLNCTARTELNVGIDFNWEYPSSKHQHKKLVNRDLKTQSGSEMKKFLSTLTIDGVTRSDQGLYTCAASSGLMTKKNSTFVRVHEKDKTHTCPPCPAPELLGGPSVFLFPPKPKDTLMISRTPEVTCVVVDVSHEDPEVKFNWYVDGVEVHNAKTKPREEQYNSTYRVVSVLTVLHQDWLNGKEYKCKVSNKALPAPIEKTISKAKGQPREPQVYTLPPSRDELTKNQVSLTCLVKGFYPSDIAVEWESNGQPENNYKTTPPVLDSDGSFFLYSKLTVDKSRWQQGNVFSCSVMHEALHNHYTQKSLSLSPG

SEQ ID NO: 6 - protein, 205 aa, synthetic construct
  source 1..205: note; note (original language) = VEGFA binding domain
SDTGRPFVEMYSEIPEIIHMTEGRELVIPCRVTSPNITVTLKKFPLDTLIPDGKRIIWDSRKGFIISNATYKEIGLLTCEATVNGHLYKTNYLTHRQTNTIIDVVLSPSHGIELSVGEKLVLNCTARTELNVGIDFNWEYPSSKHQHKKLVNRDLKTQSGSEMKKFLSTLTIDGVTRSDQGLYTCAASSGLMTKKNSTFVRVHEK

SEQ ID NO: 7 - protein, 226 aa, Homo sapiens
DKTHTCPPCPAPELLGGPSVFLFPPKPKDTLMISRTPEVTCVVVDVSHEDPEVKFNWYVDGVEVHNAKTKPREEQYNSTYRVVSVLTVLHQDWLNGKEYKCKVSNKALPAPIEKTISKAKGQPREPQVYTLPPSRDELTKNQVSLTCLVKGFYPSDIAVEWESNGQPENNYKTTPPVLDSDGSFFLYSKLTVDKSRWQQGNVFSCSVMHEALHNHYTQKSLSLSPG

SEQ ID NO: 8 - protein, 564 aa, synthetic construct
  source 1..564: note; note (original language) = first polypeptide chain and second polypeptide chain
SDTGRPFVEMYSEIPEIIHMTEGRELVIPCRVTSPNITVTLKKFPLDTLIPDGKRIIWDSRKGFIISNATYKEIGLLTCEATVNGHLYKTNYLTHRQTNTIIDVVLSPSHGIELSVGEKLVLNCTARTELNVGIDFNWEYPSSKHQHKKLVNRDLKTQSGSEMKKFLSTLTIDGVTRSDQGLYTCAASSGLMTKKNSTFVRVHEKDKTHTCPPCPAPELLGGPSVFLFPPKPKDTLMISRTPEVTCVVVDVSHEDPEVKFNWYVDGVEVHNAKTKPREEQYNSTYRVVSVLTVLHQDWLNGKEYKCKVSNKALPAPIEKTISKAKGQPREPQVYTLPPSRDELTKNQVSLTCLVKGFYPSDIAVEWESNGQPENNYKTTPPVLDSDGSFFLYSKLTVDKSRWQQGNVFSCSVMHEALHNHYTQKSLSLSPGGGGGSGGGGSGGGGSEVQLVESGGGLVQPGGSLRLSCAASGSSFSPYAMGWYRQAPGKQRELVSATSSGGFTLYADSVKGRFTISRDNSKNTVYLQMNSLRAEDTAVYYCYTYYREYDPEMYWGQGTQVTVSS

SEQ ID NO: 9 - protein, 537 aa, synthetic construct
  source 1..537: note = OPT-302
YSMTPPTLNITEESHVIDTGDSLSISCRGQHPLEWAWPGAQEAPATGDKDSEDTGVVRDCEGTDARPYCKVLLLHEVHAQDTGSYVCYYKYIKARIEGTTAASSYVFVRDFEQPFINKPDTLLVNRKDAMWVPCLVSIPGLNVTLRSQSSVLWPDGQEVVWDDRRGMLVSTPLLHDALYLQCETTWGDQDFLSNPFLVHITGNELYDIQLLPRKSLELLVGEKLVLNCTVWAEFNSGVTFDWDYPGKQAERGKWVPERRSQQTHTELSSILTIHNVSQHDLGSYVCKANNGIQRFRESTEVIVHEEPKSCDKTHTCPPCPAPELLGGPSVFLFPPKPKDTLMISRTPEVTCVVVDVSHEDPEVKFNWYVDGVEVHNAKTKPREEQYNSTYRVVSVLTVLHQDWLNGKEYKCKVSNKALPAPIEKTISKAKGQPREPQVYTLPPSRDELTKNQVSLTCLVKGFYPSDIAVEWESNGQPENNYKTTPPVLDSDGSFFLYSKLTVDKSRWQQGNVFSCSVMHEALHNHYTQKSLSLSPGK

SEQ ID NO: 10 - protein, 434 aa, synthetic construct
  source 1..434: note = IBI304
PFVEMYSEIPEIIHMTEGRELVIPCRVTSPNITVTLKKFPLDTLIPDGKRIIWDSRKGFIISNATYKEIGLLTCEATVNGHLYKTNYLTHRQTVVLSPSHGIELSVGEKLVLNCTARTELNVGIDFNWEYPSSKHQHKKLVNRDLKTQSGSEMKKFLSTLTIDGVTRSDQGLYTCAASSGLMTKKNSTFVRVHEKGGGGGGGGGGGGDKTHTCPLCPAPELLGGPSVFLFPPKPKDTLMISRTPEVTCVVVDVSHEDPEVKFNWYVDGVEVHNAKTKPREEQYNSTYRVVSVLTVLHQDWLNGKEYKCKVSNKALPAPIEKTISKAKGQPREPQVYTLPPSRDELTKNQVSLTCLVKGFYPSDIAVEWESNGQPENNYKATPPVLDSDGSFFLYSKLTVDKSRWQQGNVFSCSVMHEALHNHYTQKSLSLSPGK